European Patent Application EP 4 786 577 A1, published August 5, 2026. Title: 一种具有减肥功能的植物乳植杆菌菌株、益生菌制剂及其制备方法和用途. Applicant: 科郦有限公司. The sequence listing filed with the application follows.

SEQUENCE LISTING (11 sequences)

SEQ ID NO: 1 - DNA, 1440 bp, Lactiplantibacillus plantarum HOM2217
  source 1..1440: mol_type = other DNA
  misc_feature 1..1440: note = 16S rRNA gene
tatacatgcagtcgaacgaactctggtattgattggtgcttgcatcatgatttacatttgagtgagtggcgaactggtgagtaacacgtgggaaacctgcccagaagcgggggataacacctggaaacagatgctaataccgcataacaacttggaccgcatggtccgagtttgaaagatggcttcggctatcacttttggatggtcccgcggcgtattagctagatggtggggtaatggctcaccatggcaatgatacgtagccgacctgagagggtaatcggccacattgggactgagacacggcccaaactcctacgggaggcagcagtagggaatcttccacaatggacgaaagtctgatggagcaacgccgcgtgagtgaagaagggtttcggctcgtaaaactctgttgttaaagaagaacatatctgagagtaactgttcaggtattgacggtatttaaccagaaagccacggctaactacgtgccagcagccgcggtaatacgtaggtggcaagcgttgtccggatttattgggcgtaaagcgagcgcaggcggttttttaagtctgatgtgaaagccttcggctcaaccgaagaagtgcatcggaaactgggaaacttgagtgcagaagaggacagtggaactccatgtgtagcggtgaaatgcgtagatatatggaagaacaccagtggcgaaggcggctgtctggtctgtaactgacgctgaggctcgaaagtatgggtagcaaacaggattagataccctggtagtccataccgtaaacgatgaatgctaagtgttggagggtttccgcccttcagtgctgcagctaacgcattaagcattccgcctggggagtacggccgcaaggctgaaactcaaaggaattgacgggggcccgcacaagcggtggagcatgtggtttaattcgaagctacgcgaagaaccttaccaggtcttgacatactatgcaaatctaagagattagacgttcccttcggggacatggatacaggtggtgcatggttgtcgtcagctcgtgtcgtgagatgttgggttaagtcccgcaacgagcgcaacccttattatcagttgccagcattaagttgggcactctggtgagactgccggtgacaaaccggaggaaggtggggatgacgtcaaatcatcatgccccttatgacctgggctacacacgtgctacaatggatggtacaacgagttgcgaactcgcgagagtaagctaatctcttaaagccattctcagttcggattgtaggctgcaactcgcctacatgaagtcggaatcgctagtaatcgcggatcagcatgccgcggtgaatacgttcccgggccttgtacacaccgcccgtcacaccatgagagtttgtaacacccaaagtcggtggggtaaccttttaggaaccagccgc

SEQ ID NO: 2 - DNA, 10 bp, synthetic construct
  source 1..10: mol_type = other DNA
  misc_feature 1..10: note = OPA-02 primer
tgccgagctg

SEQ ID NO: 3 - DNA, 10 bp, synthetic construct
  source 1..10: mol_type = other DNA
  misc_feature 1..10: note = OPA-18 primer
aggtgaccgt

SEQ ID NO: 4 - DNA, 10 bp, synthetic construct
  source 1..10: mol_type = other DNA
  misc_feature 1..10: note = OPL-07 primer
aggcgggaac

SEQ ID NO: 5 - DNA, 10 bp, synthetic construct
  source 1..10: mol_type = other DNA
  misc_feature 1..10: note = OPL-16 primer
aggttgcagg

SEQ ID NO: 6 - DNA, 10 bp, synthetic construct
  source 1..10: mol_type = other DNA
  misc_structure 1..10: note = OPM-05 primer
gggaacgtgt

SEQ ID NO: 7 - DNA, 18 bp, synthetic construct
  source 1..18: mol_type = other DNA
  misc_feature 1..18: note = 27F primer
agtttgatcmtggctcag

SEQ ID NO: 8 - DNA, 19 bp, synthetic construct
  source 1..19: mol_type = other DNA
  misc_feature 1..19: note = 1492R primer
ggttaccttgttacgactt

SEQ ID NO: 9 - DNA, 452 bp, Lactiplantibacillus plantarum HOM2217
  source 1..452: mol_type = other DNA
  misc_feature 1..395: note = pheS gene
caccatattcttctggatcaatgccagacatttctaacacgtgggggtgaaccatgccggcacccagtacttcgatccaacccgtttgcttacagattgcacagcccttgccattgcaattaaagcaagttacatcagcttctacggatggttccgtgaatggaaagaagcttggccgtagccgaacatcgaattgatcgccaaacaaagtcttggcaaccagaattaaggtgcccttcaaatcagccatcgtaatatgcttgtccacgactaacccttcaatttgatgaaattgatgggaatgagttgcatcatccgtatcacgccgataaacgcggccaggtgacaagaccttcagcggtcctttagaaaaatcgtgattttcaagtgaccgcggctgatcagcagacgtctgcgtgcgtagtagcacgtctttggtaatatagaacgtg

SEQ ID NO: 10 - DNA, 1567 bp, Lactiplantibacillus plantarum S1-6
  source 1..1567: mol_type = other DNA
  misc_feature 1..1567: note = 16S rRNA gene
taatttgagagtttgatcctggctcaggacgaacgctggcggcgtgcctaatacatgcaagtcgaacgaactctggtattgattggtgcttgcatcatgatttacatttgagtgagtggcgaactggtgagtaacacgtgggaaacctgcccagaagcgggggataacacctggaaacagatgctaataccgcataacaacttggaccgcatggtccgagtttgaaagatggcttcggctatcacttttggatggtcccgcggcgtattagctagatggtggggtaacggctcaccatggcaatgatacgtagccgacctgagagggtaatcggccacattgggactgagacacggcccaaactcctacgggaggcagcagtagggaatcttccacaatggacgaaagtctgatggagcaacgccgcgtgagtgaagaagggtttcggctcgtaaaactctgttgttaaagaagaacatatctgagagtaactgttcaggtattgacggtatttaaccagaaagccacggctaactacgtgccagcagccgcggtaatacgtaggtggcaagcgttgtccggatttattgggcgtaaagcgagcgcaggcggttttttaagtctgatgtgaaagccttcggctcaaccgaagaagtgcatcggaaactgggaaacttgagtgcagaagaggacagtggaactccatgtgtagcggtgaaatgcgtagatatatggaagaacaccagtggcgaaggcggctgtctggtctgtaactgacgctgaggctcgaaagtatgggtagcaaacaggattagataccctggtagtccataccgtaaacgatgaatgctaagtgttggagggtttccgcccttcagtgctgcagctaacgcattaagcattccgcctggggagtacggccgcaaggctgaaactcaaaggaattgacgggggcccgcacaagcggtggagcatgtggtttaattcgaagctacgcgaagaaccttaccaggtcttgacatactatgcaaatctaagagattagacgttcccttcggggacatggatacaggtggtgcatggttgtcgtcagctcgtgtcgtgagatgttgggttaagtcccgcaacgagcgcaacccttattatcagttgccagcattaagttgggcactctggtgagactgccggtgacaaaccggaggaaggtggggatgacgtcaaatcatcatgccccttatgacctgggctacacacgtgctacaatggatggtacaacgagttgcgaactcgcgagagtaagctaatctcttaaagccattctcagttcggattgtaggctgcaactcgcctacatgaagtcggaatcgctagtaatcgcggatcagcatgccgcggtgaatacgttcccgggccttgtacacaccgcccgtcacaccatgagagtttgtaacacccaaagtcggtggggtaaccttttaggaaccagccgcctaaggtgggacagatgattagggtgaagtcgtaacaaggtagccgtaggagaacctgcggctggatcacctccttt

SEQ ID NO: 11 - DNA, 1512 bp, Lactiplantibacillus plantarum S2-13
  source 1..1512: mol_type = other DNA
  misc_feature 1..1512: note = 16S rRNA gene
ctggctcaggacgaacgctggcggcgtgcctaatacatgcaagtcgaacgaactctggtattgattggtgcttgcatcatgatttacatttgagtgagtggcgaactggtgagtaacacgtgggaaacctgcccagaagcgggggataacacctggaaacagatgctaataccgcataacaacttggaccgcatggtccgagtttgaaagatggcttcggctatcacttttggatggtcccgcggcgtattagctagatggtggggtaacggctcaccatggcaatgatacgtagccgacctgagagggtaatcggccacattgggactgagacacggcccaaactcctacgggaggcagcagtagggaatcttccacaatggacgaaagtctgatggagcaacgccgcgtgagtgaagaagggtttcggctcgtaaaactctgttgttaaagaagaacatatctgagagtaactgttcaggtattgacggtatttaaccagaaagccacggctaactacgtgccagcagccgcggtaatacgtaggtggcaagcgttgtccggatttattgggcgtaaagcgagcgcaggcggttttttaagtctgatgtgaaagccttcggctcaaccgaagaagtgcatcggaaactgggaaacttgagtgcagaagaggacagtggaactccatgtgtagcggtgaaatgcgtagatatatggaagaacaccagtggcgaaggcggctgtctggtctgtaactgacgctgaggctcgaaagtatgggtagcaaacaggattagataccctggtagtccataccgtaaacgatgaatgctaagtgttggagggtttccgcccttcagtgctgcagctaacgcattaagcattccgcctggggagtacggccgcaaggctgaaactcaaaggaattgacgggggcccgcacaagcggtggagcatgtggtttaattcgaagctacgcgaagaaccttaccaggtcttgacatactatgcaaatctaagagattagacgttcccttcggggacatggatacaggtggtgcatggttgtcgtcagctcgtgtcgtgagatgttgggttaagtcccgcaacgagcgcaacccttattatcagttgccagcattaagttgggcactctggtgagactgccggtgacaaaccggaggaaggtggggatgacgtcaaatcatcatgccccttatgacctgggctacacacgtgctacaatggatggtacaacgagttgcgaactcgcgagagtaagctaatctcttaaagccattctcagttcggattgtaggctgcaactcgcctacatgaagtcggaatcgctagtaatcgcggatcagcatgccgcggtgaatacgttcccgggccttgtacacaccgcccgtcacaccatgagagtttgtaacacccaaagtcggtggggtaaccttttaggaaccagccgcctaaggtgggacagatgattagggtgaagtcgtaacaagg